European Patent Application EP 4 621 061 A1, published September 24, 2025. Title: METHOD FOR PRODUCING PSICOSE BY FERMENTATION AND ISOMERIZATION OF BACILLUS SUBTILIS. Applicant: ANHUI JINHE INDUSTRIAL CO., LTD. The sequence listing filed with the application follows.

SEQUENCE LISTING (16 sequences)

SEQ ID NO: 1 - DNA, 27 bp, synthetic construct
  source 1..27: mol_type = other DNA
tacaaagcaaaagcgaaaatgaccatc

SEQ ID NO: 2 - DNA, 36 bp, synthetic construct
  source 1..36: mol_type = other DNA
atgctatacgaacggtacttagaagagagaaggtaa

SEQ ID NO: 3 - DNA, 36 bp, synthetic construct
  source 1..36: mol_type = other DNA
ttaccttctctcttctaagtaccgttcgtatagcat

SEQ ID NO: 4 - DNA, 36 bp, synthetic construct
  source 1..36: mol_type = other DNA
caagcaaagctgttttatctaccgttcgtataatgt

SEQ ID NO: 5 - DNA, 36 bp, synthetic construct
  source 1..36: mol_type = other DNA
acattatacgaacggtagataaaacagctttgcttg

SEQ ID NO: 6 - DNA, 26 bp, synthetic construct
  source 1..26: mol_type = other DNA
cagctgataggattcttgctcgctta

SEQ ID NO: 7 - DNA, 50 bp, synthetic construct
  source 1..50: mol_type = other DNA
cgtctgtacgttccttaaggaattcttaggagtgtttatgacattctaat

SEQ ID NO: 8 - DNA, 50 bp, synthetic construct
  source 1..50: mol_type = other DNA
tagaatgcaaaaagtgaaatcataatgataggtggtatgttttcgcttga

SEQ ID NO: 9 - DNA, 50 bp, synthetic construct; identical to SEQ ID NO: 8
  source 1..50: mol_type = other DNA

SEQ ID NO: 10 - DNA, 47 bp, synthetic construct
  source 1..47: mol_type = other DNA
tcaagcgaaaacataccacctatcattatgatttcactttttgcatt

SEQ ID NO: 11 - DNA, 50 bp, synthetic construct
  source 1..50: mol_type = other DNA
attaacttacctaaatggagaattcaatctattattaatctgttcagcaa

SEQ ID NO: 12 - DNA, 50 bp, synthetic construct
  source 1..50: mol_type = other DNA
caccatttcctctttagaaagatcttcccttttcagataattttagattt

SEQ ID NO: 13 - DNA, 50 bp, synthetic construct
  source 1..50: mol_type = other DNA
aaatctaaaattatctgaaaagggaagatctttctaaagaggaaatggtg

SEQ ID NO: 14 - DNA, 50 bp, synthetic construct
  source 1..50: mol_type = other DNA
ttgctgaacagattaataatagattgaattctccatttaggtaagttaat

SEQ ID NO: 15 - DNA, 818 bp, synthetic construct
  source 1..818: mol_type = other DNA
tacaaagcaaaagcgaaaatgaccatcgagacagggagtgagcctcaagtatacaatgtggaaatctggcacaaaaagccgtctctgtacagggtttatttagaaaatccgaaaaaggaccaaaaccaagtcattttacgaaatgaaaacggagtattcgttctcacgccgtctttaaataagagcttcagatttcaaagcgattggccgaacaacagcagccaggtttatctgtttgaatcgctcgtaaaggatgttcaaaacgattcggatgcagttttcacagcgaaagaaaagaaatacgtatttgaaacaaaaacaaactatcagcataacaaaatgctgcccacgcaagaaatcacatttaacaaaaaagatatgagcccgtcatctgtcaaagtgatggatactgaccggaaagtgatggtcaaagtagaattcagcagctttgaatttaataaacaatttgataaagaatcatttgatgaaaagaaaaatatgaccctttctcaaatggatgtcgccacaagcgcaaagccttccgatacatttgcggtcaaaacgccgctggaactgccgcttggcgtcaagctgcttgaagaaaaagatatatctactgaagacgggaagcgcatcatcatgacgtacggaggagaaaaatcatttacgttaattcaggaaaaagcccagattgccaaggcttcctcctccgttacgctgaacggcgaaccggtaaatctcggctacaccatcggcgccctgtcggatgcatcattatcatggacatatgacggcgtagattaccttctctcttctaa

SEQ ID NO: 16 - DNA, 957 bp, synthetic construct
  source 1..957: mol_type = other DNA
ataaaacagctttgcttgaagagtgaataatggtatcattatcactggatggataaaagagtcgtatccgtaagtttggtggaggtgtatgttttttgtctgaatccagcgcaagaaccgaaatgaaaatcagcttgcccgaaaacctagtagctgaattggatggtgtagcgatgcgggagaaacgaagcagaaacgaactgatatcacaagcagtgagagcgtatgtcagcgaacgaacaactcgtcacaaccgtgatttgatgagacgcggctatatggaaatggcgaaaatcaacctgaatatttcttctgaggctcactttgcggagtgcgaggctgaaacgacagttgagcgcttagtcagcggaggataatcatttgattgtgaaacgcggcgatgtttattttgctgatttatctcctgttgttggctcagagcaaggcggggtgcgcccggttttagtgatccaaaatgacatcggaaatcgcttcagcccaactgctattgttgcagccataacagcacaaatacagaaagcgaaattaccaacccacgtcgaaatcgatgcaaaacgctacggttttgaaagagattccgttattttgctggagcaaattcggacgattgacaagcaaaggttaacggataagattactcatctggatgatgaaatgatggataaggttgatgaagccttacaaatcagtttggcactcattgatttttagacatatttgcaggttgctcaaatagagcaactttttttgttttcaaaaaacataaacgatataatagtgaaataacgaaaaaatatgttgttttttattgggaggtaagcgaatttgatgtcgaaccagactgtataccagttcattgccgaaaatcaaaatgaactgctccaactgtggactgacacactaaaagaattaagcgagcaagaatcctatcagctg